European Patent Application EP 4 327 833 A1, published February 28, 2024. Title: Radioactive antitumor agent. Applicant: NIHON MEDI-PHYSICS CO., LTD. Sumitomo Pharma Co., Ltd. The sequence listing filed with the application follows.

SEQUENCE LISTING (26 sequences)

SEQ ID NO: 1 - protein, 121 aa, Artificial Sequence
  Humanaized antibody heavy chain variable region 1 (H01)
EVQLLESGGGLVQPGGSLRLSCAASGFTFSNYGMSWVRQAPGKGLEWVSTISNSGRYTYFPDSVKGRFTISRDNSKNTLYLQMNSLRAEDTALYYCTRHLDYANYDAMDYWGQGTLVTVSS

SEQ ID NO: 2 - protein, 121 aa, Artificial Sequence
  Humanaized antibody heavy chain variable region 2 (H02)
LVQLVESGGGVVRPGGSLRLSCAASGFTFSNYGMSWIRQAPGKGLEWVSTISNSGRYTYFPDSVKGRFTISRDNAKNSLYLQMNSLRAEDTALYYCTRHLDYANYDAMDYWGQGTLVTVSS

SEQ ID NO: 3 - protein, 121 aa, Artificial Sequence
  Humanaized antibody heavy chain variable region 3 (H03)
LVQLVESGGGVVQPGRSLRLSCAASGFTFSNYGMSWVRQAPGKGLEWVATISNSGRYTYFPDSVKGRFTISRDNSKNTLYLQMNSLRAEDTAVYYCTRHLDYANYDAMDYWGQGTLVTVSS

SEQ ID NO: 4 - protein, 121 aa, Artificial Sequence
  Humanaized antibody heavy chain variable region 4 (H04)
EVQLLESGGGLVQPGGSLRLSCAVSGFTFSNYGMSWVRQAPGKGLEWVSTISNSGRYTYFPDSVKGRFTISRDNSRNTLYLQMNTLRAEDTAVYYCTRHLDYANYDAMDYWGQGTPVTVSS

SEQ ID NO: 5 - protein, 111 aa, Artificial Sequence
  Humanaized antibody light chain variable region 1 (L01)
DIVMTQSPSSLSASVGDRVTITCRASKSVTTSDFSYMHWYQQKPGKAPKLLIYLASNLESGVPSRFSGSGSGTDFTLTISSLQPEDFATYYCQHSREFPWTFGGGTKVEIK

SEQ ID NO: 6 - protein, 111 aa, Artificial Sequence
  Humanaized antibody light chain variable region 2 (L02)
DVVMTQSPSTLSASVGDRVTITCRASKSVTTSDFSYMHWYQQKPGQAPKLLIYLASNLESGVPSRFSGSGSGTDFTLTISSLQPEDFATYYCQHSREFPWTFGQGTKLEIK

SEQ ID NO: 7 - protein, 111 aa, Artificial Sequence
  Humanaized antibody light chain variable region 3 (L03)
DIQMTQSPSSLSASVGDRVTITCRASKSVTTSDFSYMHWYQQKPGKSPKLLIYLASNLESGVPSRFSGSGSGTDFSLTISSLQPEDFATYYCQHSREFPWTFGGGTKVEIK

SEQ ID NO: 8 - protein, 111 aa, Artificial Sequence
  Humanaized antibody light chain variable region 4 (L04)
DIVMTQSPDSLAVSLGERATINCKASKSVTTSDFSYLHWYQQKPGQPPKLLIYLASNLESGVPDRFSGSGSGTDFTLTISSLQAEDVAVYYCQHSREFPWTFGGGTKLEIK

SEQ ID NO: 9 - protein, 13 aa, Artificial
  antibody-binding peptide
  misc_feature (6)..(6): Xaa is lysine, cystein, aspartic acid, glutamic acid, 2-amino suberic acid, or diaminopropionic acid
DCAYHXGELVWCT

SEQ ID NO: 10 - protein, 17 aa, Artificial
  antibody-binding peptide
  misc_feature (8)..(8): Xaa is lysine, cystein, aspartic acid, glutamic acid, 2-amino suberic acid, or diaminopropionic acid
GPDCAYHXGELVWCTFH

SEQ ID NO: 11 - protein, 13 aa, Artificial
  antibody-binding peptide
  misc_feature (6)..(6): Xaa is lysine, cystein, aspartic acid, glutamic acid, 2-amino suberic acid, or diaminopropionic acid
RCAYHXGELVWCS

SEQ ID NO: 12 - protein, 17 aa, Artificial
  antibody-binding peptide
  misc_feature (8)..(8): Xaa is lysine, cystein, aspartic acid, glutamic acid, 2-amino suberic acid, or diaminopropionic acid
GPRCAYHXGELVWCSFH

SEQ ID NO: 13 - protein, 17 aa, Artificial
  antibody-binding peptide
  misc_feature (8)..(8): Xaa is lysine, cystein, aspartic acid, glutamic acid, 2-amino suberic acid, or diaminopropionic acid
SPDCAYHXGELVWCTFH

SEQ ID NO: 14 - protein, 17 aa, Artificial
  antibody-binding peptide
  misc_feature (8)..(8): Xaa is lysine, cystein, aspartic acid, glutamic acid, 2-amino suberic acid, or diaminopropionic acid
GDDCAYHXGELVWCTFH

SEQ ID NO: 15 - protein, 17 aa, Artificial
  antibody-binding peptide
  misc_feature (8)..(8): Xaa is lysine, cystein, aspartic acid, glutamic acid, 2-amino suberic acid, or diaminopropionic acid
GPSCAYHXGELVWCTFH

SEQ ID NO: 16 - protein, 17 aa, Artificial
  antibody-binding peptide
  misc_feature (8)..(8): Xaa is lysine, cystein, aspartic acid, glutamic acid, 2-amino suberic acid, or diaminopropionic acid
GPDCAYHXGELVWCSFH

SEQ ID NO: 17 - protein, 17 aa, Artificial
  antibody-binding peptide
  misc_feature (8)..(8): Xaa is lysine, cystein, aspartic acid, glutamic acid, 2-amino suberic acid, or diaminopropionic acid
GPDCAYHXGELVWCTHH

SEQ ID NO: 18 - protein, 17 aa, Artificial
  antibody-binding peptide
  misc_feature (8)..(8): Xaa is lysine, cystein, aspartic acid, glutamic acid, 2-amino suberic acid, or diaminopropionic acid
GPDCAYHXGELVWCTFY

SEQ ID NO: 19 - protein, 17 aa, Artificial
  antibody-binding peptide
  misc_feature (8)..(8): Xaa is lysine, cystein, aspartic acid, glutamic acid, 2-amino suberic acid, or diaminopropionic acid
SPDCAYHXGELVWCTFY

SEQ ID NO: 20 - protein, 17 aa, Artificial
  antibody-binding peptide
  misc_feature (8)..(8): Xaa is lysine, cystein, aspartic acid, glutamic acid, 2-amino suberic acid, or diaminopropionic acid
SDDCAYHXGELVWCTFY

SEQ ID NO: 21 - protein, 17 aa, Artificial
  antibody-binding peptide
  misc_feature (8)..(8): Xaa is lysine, cystein, aspartic acid, glutamic acid, 2-amino suberic acid, or diaminopropionic acid
RGNCAYHXGQLVWCTYH

SEQ ID NO: 22 - protein, 17 aa, Artificial
  antibody-binding peptide
  misc_feature (2)..(2): Xaa is homocysteine
  misc_feature (8)..(8): Xaa is lysine, cystein, aspartic acid, glutamic acid, 2-amino suberic acid, or diaminopropionic acid
  misc_feature (16)..(16): Xaa is homocysteine
GXDCAYHXGELVWCTXH

SEQ ID NO: 23 - protein, 121 aa, Artificial Sequence
  Kimeric antibody heavy chain variable region 7 (H07)
EVKLVESGGVLVKSGGSLKLSCAVSGFTFSNYGMSWVRQTPEKRLEWVATISNSGRYTYFPDSVKGPFAISRDNAKNNLYLQMSSLRSADTALYYCTRHLDYANYDAMDYWGQGTSVTVSS

SEQ ID NO: 24 - protein, 111 aa, Artificial Sequence
  Kimeric antibody light chain variable region 8 (L08)
DIVLTQSPASLAVSLGQRATISCRASKSVTTSDFSYMHWYQQKPGQPPKLLLYLASNLESGVPDRFSGSGSGYDFYLNIHPVEEEDAATYYCQHSREFPWTFGGGTKLEIK

SEQ ID NO: 25 - protein, 330 aa, Artificial Sequence [sequence omitted]

SEQ ID NO: 26 - protein, 107 aa, Artificial Sequence [sequence omitted]